European Patent Specification EP 3 692 140 B1, published July 19, 2023. Title: METHODS FOR SELECTIVELY EXPANDING CELLS EXPRESSING A TCR WITH A MURINE CONSTANT REGION. Applicant: THE UNITED STATES OF AMERICA, AS REPRESENTED BY THE SECRETARY, DEPARTMENT OF HEALTH AND HUMAN SERVICES. The sequence listing filed with the application follows.

SEQUENCE LISTING (6 sequences)

SEQ ID NO: 1 - protein, 173 aa, Mus musculus
EDLRNVTPPKVSLFEPSKAEIANKQKATLVCLARGFFPDHVELSWWVNGKEVHSGVSTDPQAYKESNYSYCLSSRLRVSATFWHNPRNHFRCQVQFHGLSEEDKWPEGSPKPVTQNISAEAWGRADCGITSASYQQGVLSATILYEILLGKATLYAVLVSTLVVMAMVKRKNS

SEQ ID NO: 2 - protein, 109 aa, Mus musculus
DLRNVTPPKVSLFEPSKAEIANKQKATLVCLARGFFPDHVELSWWVNGKEVHSGVSTDPQAYKESNYSYCLSSRLRVSATFWHNPRNHFRCQVQFHGLSEEDKWPEGSP

SEQ ID NO: 3 - protein, 121 aa, Armenian hamster
EVYLVESGGDLVQPGSSLKVSCAASGFTFSDFWMYWVRQAPGKGLEWVGRIKNIPNNYATEYADSVRGRFTISRDDSRNSIYLQMNRLRVDDTAIYYCTRAGRFDHFDYWGQGTMVTVSSA

SEQ ID NO: 4 - protein, 110 aa, Armenian hamster
YELIQPSSASVTVGETVKITCSGDQLPKNFAYWFQQKSDKNILLLIYMDNKRPSGIPERFSGSTSGTTATLTISGAQPEDEAAYYCLSSYGDNNDLVFGSGTQLTVLRGP

SEQ ID NO: 5 - protein, 222 aa, Armenian hamster
EVYLVESGGDLVQPGSSLKVSCAASGFTFSDFWMYWVRQAPGKGLEWVGRIKNIPNNYATEYADSVRGRFTISRDDSRNSIYLQMNRLRVDDTAIYYCTRAGRFDHFDYWGQGTMVTVSSATTTAPSVYPLAPACDSTTSTTDTVTLGCLVKGYFPEPVTVSWNSGALTSGVHTFPSVLHSGLYSLSSSVTVPSSTWPKQPITCNVAHPASSTKVDKKIEPR

SEQ ID NO: 6 - protein, 212 aa, Armenian hamster
YELIQPSSASVTVGETVKITCSGDQLPKNFAYWFQQKSDKNILLLIYMDNKRPSGIPERFSGSTSGTTATLTISGAQPEDEAAYYCLSSYGDNNDLVFGSGTQLTVLRGPKSSPKVTVFPPSPEELRTNKATLVCLVNDFYPGSATVTWKANGATINDGVKTTKPSKQGQNYMTSSYLSLTADQWKSHNRVSCQVTHEGETVEKSLSPAECL